European Patent Application EP 4 345 104 A1, published April 3, 2024. Title: Method for preparing liraglutide. Applicant: Bachem Holding AG. The sequence listing filed with the application follows.

SEQUENCE LISTING (4 sequences)

SEQ ID NO: 1 - protein, 31 aa, synthetic construct
HAEGTFTSDVSSYLEGQAAKEFIAWLVRGRG

SEQ ID NO: 2 - protein, 31 aa, synthetic construct
  SITE 20: note = lysyl(gamma-glutamate)
  SITE 1: note = trifluoroacetic acid-histidine
XAEGTFTSDVSSYLEGQAAXEFIAWLVRGRG

SEQ ID NO: 3 - protein, 31 aa, synthetic construct
  SITE 20: note = lysyl(palmitoyl-gamma-glutamyl)
HAEGTFTSDVSSYLEGQAAXEFIAWLVRGRG

SEQ ID NO: 4 - protein, 31 aa, synthetic construct; identical to SEQ ID NO: 2
  SITE 1: note = trifluoroacetic acid-histidine
  SITE 20: note = lysyl(palmitoyl-gamma-glutamyl)